European Patent Specification EP 3 907 293 B1, published August 13, 2025. Title: Biochip, method of preparation and use thereof. Applicant: BGI SHENZHEN BGI SHENZHEN CO., LTD. Application EP19896991.7. The sequence listing filed with the application follows.

SEQUENCE LISTING (16 sequences)

SEQ ID NO: 1 - DNA, 59 bp, Artificial Sequence
gcccatttctcgaacgtacttctcacagtttcagttaagaaatcgaagaagtaagatac

SEQ ID NO: 2 - DNA, 59 bp, Artificial Sequence
agtacgttcgagaaatgggccactaccggagaaacacttcagttactctttgagatgaa

SEQ ID NO: 3 - DNA, 59 bp, Artificial Sequence
aagtatttgcataagcactttaaatgtaggttttttcatctcaaagagtaactgaagtg

SEQ ID NO: 4 - DNA, 59 bp, Artificial Sequence
acatttaaagtgcttatgcaaatacttataggtggcaatcaagttgaaaatgaattgct

SEQ ID NO: 5 - DNA, 59 bp, Artificial Sequence
caaatcggaaattgttctccttgaacaaagcgtcaagcaattcattttcaacttgattg

SEQ ID NO: 6 - DNA, 59 bp, Artificial Sequence
caaggagaacaatttccgatttgctggtcttcgtagcatgcccctcgatttccccggat

SEQ ID NO: 7 - DNA, 59 bp, Artificial Sequence
aactatttctcctcgacccttcattgccctgttgtaagtagatccggggaaatcgaggg

SEQ ID NO: 8 - DNA, 59 bp, Artificial Sequence
gaagggtcgaggagaaatagttaagatatacgaacggataataaatgaaagaaaagtga

SEQ ID NO: 9 - DNA, 59 bp, Artificial Sequence
ggtccttggctctcctctagtcttggcaatcatcacttttctttcatttattatccgtt

SEQ ID NO: 10 - DNA, 59 bp, Artificial Sequence
tagaggagagccaaggaccaacatactggatataatgctagacagtcaatgtgatgagg

SEQ ID NO: 11 - DNA, 59 bp, Artificial Sequence
actttcatgatattctcatcattcaatacttttccttcctcatcacattgactgtctag

SEQ ID NO: 12 - DNA, 59 bp, Artificial Sequence
gtattgaatgatgagaatatcatgaaagtgctgctttggtatacatttagtggttatga

SEQ ID NO: 13 - DNA, 59 bp, Artificial Sequence
ataatagtctgtgtggcaacctttgcaatagattcataaccactaaatgtataccaaag

SEQ ID NO: 14 - DNA, 59 bp, Artificial Sequence
aggttgccacacagactattatgttattggaaaaacaccccgagtgcttccagaaagca

SEQ ID NO: 15 - DNA, 5 bp, Artificial Sequence
ttttt

SEQ ID NO: 16 - DNA, 30 bp, Artificial Sequence
tttttttttttttttttttttttttttttt